European Patent Application EP 4 375 368 A1, published May 29, 2024. Title: RECOMBINANT VIRUS CONTAINING DEGRON, PREPARATION METHOD THEREFOR, AND APPLICATION THEREOF. Applicant: SHENZHEN INSTITUTES OF ADVANCED TECHNOLOGY CHINESE ACADEMY OF SCIENCES. Application EP 22855319.4, filed August 4, 2022. The sequence listing filed with the application follows.

SEQUENCE LISTING (112 sequences)

SEQ ID NO: 1 - protein, 7 aa, synthetic construct
  REGION 1..7: note = Degron1
ALAPYIP

SEQ ID NO: 2 - protein, 10 aa, synthetic construct
  REGION 1..10: note = Degron2
DRHDSGLDSM

SEQ ID NO: 3 - protein, 40 aa, synthetic construct
  REGION 1..40: note = Degron
SHGFPPEVEEQDDGTLPMSCAQESGMDRHPAACASARINV

SEQ ID NO: 4 - protein, 30 aa, synthetic construct
  REGION 1..30: note = Degron
FVNQHLCGSHLVEALYLVCGERGFFYTPKA

SEQ ID NO: 5 - protein, 6 aa, synthetic construct
  VARIANT 4: note = X can be any amino acid
  VARIANT 5: note = X can be any amino acid
DSGXXS

SEQ ID NO: 6 - protein, 10 aa, synthetic construct
  VARIANT 7: note = X can be any amino acid
  VARIANT 8: note = X can be any amino acid
DRHDSGXXSM

SEQ ID NO: 7 - protein, 12 aa, synthetic construct
  REGION 1..12: note = Degron
LGSWRHWRGQEG

SEQ ID NO: 8 - protein, 13 aa, synthetic construct
  REGION 1..13: note = Degron
SLYKKVVGTMAAG

SEQ ID NO: 9 - protein, 12 aa, synthetic construct
  REGION 1..12: note = Degron
MLSESRNFPAQA

SEQ ID NO: 10 - protein, 12 aa, synthetic construct
  REGION 1..12: note = Degron
ERAPTGRWGRRG

SEQ ID NO: 11 - protein, 12 aa, synthetic construct
  REGION 1..12: note = Degron
KKVGRARPCQRG

SEQ ID NO: 12 - protein, 12 aa, synthetic construct
  REGION 1..12: note = Degron
APRAPRQRSRDG

SEQ ID NO: 13 - protein, 11 aa, synthetic construct
  REGION 1..11: note = Degron
SWRLTGSGMKG

SEQ ID NO: 14 - protein, 12 aa, synthetic construct
  REGION 1..12: note = Degron
WRPGRRGPSSGG

SEQ ID NO: 15 - protein, 12 aa, synthetic construct
  REGION 1..12: note = Degron
LRGPSPPPMAGG

SEQ ID NO: 16 - protein, 12 aa, synthetic construct
  REGION 1..12: note = Degron
WRPGRRGPSSGG

SEQ ID NO: 17 - protein, 12 aa, synthetic construct
  REGION 1..12: note = Degron
MALAVRVVYCGA

SEQ ID NO: 18 - protein, 12 aa, synthetic construct
  REGION 1..12: note = Degron
KKNVEAIGLLGG

SEQ ID NO: 19 - protein, 12 aa, synthetic construct
  REGION 1..12: note = Degron
PPGPPLSSPRPR

SEQ ID NO: 20 - protein, 12 aa, synthetic construct
  REGION 1..12: note = Degron
TMNNEEDLLRSL

SEQ ID NO: 21 - protein, 12 aa, synthetic construct
  REGION 1..12: note = Degron
TMEPPGGRQKKR

SEQ ID NO: 22 - protein, 12 aa, synthetic construct
  REGION 1..12: note = Degron
QERGPTWDKNLR

SEQ ID NO: 23 - protein, 12 aa, synthetic construct
  REGION 1..12: note = Degron
GTMAVLRQRPGR

SEQ ID NO: 24 - protein, 12 aa, synthetic construct
  REGION 1..12: note = Degron
LCTRSWDVTPNR

SEQ ID NO: 25 - protein, 12 aa, synthetic construct
  REGION 1..12: note = Degron
ANQPAQCRKTRI

SEQ ID NO: 26 - protein, 12 aa, synthetic construct
  REGION 1..12: note = Degron
EEARLKYDKSRI

SEQ ID NO: 27 - protein, 12 aa, synthetic construct
  REGION 1..12: note = Degron
LNDGPKPGQSRF

SEQ ID NO: 28 - protein, 12 aa, synthetic construct
  REGION 1..12: note = Degron
TSLYKKVGMGRK

SEQ ID NO: 29 - protein, 12 aa, synthetic construct
  REGION 1..12: note = Degron
YKKVGTMRGRGL

SEQ ID NO: 30 - protein, 12 aa, synthetic construct
  REGION 1..12: note = Degron
VGTMAAGRAPGK

SEQ ID NO: 31 - protein, 12 aa, synthetic construct
  REGION 1..12: note = Degron
KKVGTMRGVGYP

SEQ ID NO: 32 - protein, 12 aa, synthetic construct
  REGION 1..12: note = Degron
EGPLWHPRICGS

SEQ ID NO: 33 - protein, 12 aa, synthetic construct
  REGION 1..12: note = Degron
EMALSPPRSWGQ

SEQ ID NO: 34 - protein, 12 aa, synthetic construct
  REGION 1..12: note = Degron
RSGLRRRRHRGE

SEQ ID NO: 35 - protein, 12 aa, synthetic construct
  REGION 1..12: note = Degron
VSGIMRRPWGMN

SEQ ID NO: 36 - protein, 12 aa, synthetic construct
  REGION 1..12: note = Degron
KRVLIRVTYCGL

SEQ ID NO: 37 - protein, 12 aa, synthetic construct
  REGION 1..12: note = Degron
MALAVRVVYCGA

SEQ ID NO: 38 - protein, 35 aa, synthetic construct
  REGION 1..35: note = Degron
PSSPVQTTPLSQAVATPSRSSAAAAAALDLSGRRG

SEQ ID NO: 39 - protein, 36 aa, synthetic construct
  REGION 1..36: note = Degron
HHGKGFFGSGHYTAYCYNTEGGACALLCGVGDTERG

SEQ ID NO: 40 - protein, 35 aa, synthetic construct
  REGION 1..35: note = Degron
VAEITKQLPPVVPVSKPGALRRSLSRSMSQEAQRG

SEQ ID NO: 41 - protein, 10 aa, synthetic construct
  REGION 1..10: note = Degron
KKRPPPGLDR

SEQ ID NO: 42 - protein, 10 aa, synthetic construct
  REGION 1..10: note = Degron
SVNSLLKELR

SEQ ID NO: 43 - protein, 10 aa, synthetic construct
  REGION 1..10: note = Degron
HEWVLREGEE

SEQ ID NO: 44 - protein, 10 aa, synthetic construct
  REGION 1..10: note = Degron
EYLLKMATEE

SEQ ID NO: 45 - protein, 10 aa, synthetic construct
  REGION 1..10: note = Degron
ELCKSYRRLQ

SEQ ID NO: 46 - protein, 10 aa, synthetic construct
  REGION 1..10: note = Degron
VALKFKPRKH

SEQ ID NO: 47 - protein, 10 aa, synthetic construct
  REGION 1..10: note = Degron
GLGCKVLRRH

SEQ ID NO: 48 - protein, 6 aa, synthetic construct
  REGION 1..6: note = Degron
RHCGRT

SEQ ID NO: 49 - protein, 6 aa, synthetic construct
  REGION 1..6: note = Degron
RSHGTL

SEQ ID NO: 50 - protein, 6 aa, synthetic construct
  REGION 1..6: note = Degron
RFRGLR

SEQ ID NO: 51 - protein, 6 aa, synthetic construct
  REGION 1..6: note = Degron
RNLGIR

SEQ ID NO: 52 - protein, 10 aa, synthetic construct
  REGION 1..10: note = Degron
RGRLTRNKGP

SEQ ID NO: 53 - protein, 10 aa, synthetic construct
  REGION 1..10: note = Degron
SLFRKRNKGK

SEQ ID NO: 54 - protein, 10 aa, synthetic construct
  REGION 1..10: note = Degron
RTAASGRRWG

SEQ ID NO: 55 - protein, 10 aa, synthetic construct
  REGION 1..10: note = Degron
GLLKRPCLRG

SEQ ID NO: 56 - protein, 10 aa, synthetic construct
  REGION 1..10: note = Degron
QRKLQRTSRG

SEQ ID NO: 57 - protein, 10 aa, synthetic construct
  REGION 1..10: note = Degron
PKSKVCQQRG

SEQ ID NO: 58 - protein, 10 aa, synthetic construct
  REGION 1..10: note = Degron
KRLLKGSQYG

SEQ ID NO: 59 - protein, 12 aa, synthetic construct
  REGION 1..12: note = Degron
PHKRLLKGSQYG

SEQ ID NO: 60 - protein, 10 aa, synthetic construct
  REGION 1..10: note = Degron
KESNDCSCGG

SEQ ID NO: 61 - protein, 10 aa, synthetic construct
  REGION 1..10: note = Degron
DCVCRGSTGG

SEQ ID NO: 62 - protein, 10 aa, synthetic construct
  REGION 1..10: note = Degron
VAPRSRDERG

SEQ ID NO: 63 - protein, 10 aa, synthetic construct
  REGION 1..10: note = Degron
AHQLQALRRG

SEQ ID NO: 64 - protein, 5 aa, synthetic construct
  REGION 1..5: note = Degron
LTGKG

SEQ ID NO: 65 - protein, 6 aa, synthetic construct
  REGION 1..6: note = Degron
YYCFFG

SEQ ID NO: 66 - protein, 5 aa, synthetic construct
  REGION 1..5: note = Degron
LEKGG

SEQ ID NO: 67 - protein, 5 aa, synthetic construct
  REGION 1..5: note = Degron
AAHKG

SEQ ID NO: 68 - protein, 5 aa, synthetic construct
  REGION 1..5: note = Degron
ALRRG

SEQ ID NO: 69 - protein, 5 aa, synthetic construct
  REGION 1..5: note = Degron
GGSGG

SEQ ID NO: 70 - protein, 5 aa, synthetic construct
  REGION 1..5: note = Degron
RDERG

SEQ ID NO: 71 - protein, 5 aa, synthetic construct
  REGION 1..5: note = Degron
SRVKG

SEQ ID NO: 72 - protein, 5 aa, synthetic construct
  REGION 1..5: note = Degron
PASGG

SEQ ID NO: 73 - protein, 5 aa, synthetic construct
  REGION 1..5: note = Degron
AIHGG

SEQ ID NO: 74 - protein, 5 aa, synthetic construct
  REGION 1..5: note = Degron
GAEAG

SEQ ID NO: 75 - protein, 5 aa, synthetic construct
  REGION 1..5: note = Degron
GSTGG

SEQ ID NO: 76 - protein, 5 aa, synthetic construct
  REGION 1..5: note = Degron
RGMGG

SEQ ID NO: 77 - protein, 5 aa, synthetic construct
  REGION 1..5: note = Degron
LVHAG

SEQ ID NO: 78 - protein, 5 aa, synthetic construct
  REGION 1..5: note = Degron
SLQTG

SEQ ID NO: 79 - protein, 5 aa, synthetic construct
  REGION 1..5: note = Degron
PVPGG

SEQ ID NO: 80 - protein, 5 aa, synthetic construct
  REGION 1..5: note = Degron
NYKSG

SEQ ID NO: 81 - protein, 5 aa, synthetic construct
  REGION 1..5: note = Degron
PRKQG

SEQ ID NO: 82 - protein, 5 aa, synthetic construct
  REGION 1..5: note = Degron
TPRGG

SEQ ID NO: 83 - protein, 5 aa, synthetic construct
  REGION 1..5: note = Degron
GCSGG

SEQ ID NO: 84 - protein, 5 aa, synthetic construct
  REGION 1..5: note = Degron
EAQRG

SEQ ID NO: 85 - protein, 5 aa, synthetic construct
  REGION 1..5: note = Degron
GKAWG

SEQ ID NO: 86 - protein, 5 aa, synthetic construct
  REGION 1..5: note = Degron
PAGGG

SEQ ID NO: 87 - protein, 5 aa, synthetic construct
  REGION 1..5: note = Degron
VVLYG

SEQ ID NO: 88 - protein, 5 aa, synthetic construct
  REGION 1..5: note = Degron
LTLKG

SEQ ID NO: 89 - protein, 5 aa, synthetic construct
  REGION 1..5: note = Degron
GFQSG

SEQ ID NO: 90 - protein, 5 aa, synthetic construct
  REGION 1..5: note = Degron
RVQWG

SEQ ID NO: 91 - protein, 38 aa, synthetic construct
  REGION 1..38: note = Degron
SRTEGQFGTTQSNGTFFNGASPGTPPAPSQHQQSLTSL

SEQ ID NO: 92 - protein, 53 aa, synthetic construct
  REGION 1..53: note = Degron
YRPIPFQPEGAGEGTDEDKSNRIGNNGLRLNDGNGNGQLAPSPTPQGTEAVRA

SEQ ID NO: 93 - protein, 37 aa, synthetic construct
  REGION 1..37: note = Degron
RKFSNNPQPNAISNGTSTSERPGEGATQGIVEEEVLQ

SEQ ID NO: 94 - protein, 37 aa, synthetic construct
  REGION 1..37: note = Degron
IRTESAEEAEMASVPNGSPSWHPGASHVVNGAAGHSN

SEQ ID NO: 95 - protein, 37 aa, synthetic construct
  REGION 1..37: note = Degron
WHEIEMESGEEAMEPANETGNTLNGSPSWHPSPSHVI

SEQ ID NO: 96 - protein, 37 aa, synthetic construct
  REGION 1..37: note = Degron
NRTDFAGEEDEMDGVLNGSPSWHAATSHIVNGATVHQ

SEQ ID NO: 97 - protein, 37 aa, synthetic construct
  REGION 1..37: note = Degron
NRTDTAAEAEMDSVLNGSPSWHPPAGHVVNGATVHRS

SEQ ID NO: 98 - protein, 37 aa, synthetic construct
  REGION 1..37: note = Degron
NRTDTAAEAEMDSVLNGSPSWHPPAGHVVNGAAVHRS

SEQ ID NO: 99 - protein, 37 aa, synthetic construct
  REGION 1..37: note = Degron
NRTEVLEGAEIPSTVNGSPSWHPADSRAVSGATGHSS

SEQ ID NO: 100 - protein, 37 aa, synthetic construct
  REGION 1..37: note = Degron
NRTEAPEGTELPSTVNGSPSWHPADSRAGSGATGHSS

SEQ ID NO: 101 - protein, 37 aa, synthetic construct
  REGION 1..37: note = Degron
NRTEAPEGTESERETPSAINGNPSWHLADSPAVNGAT

SEQ ID NO: 102 - protein, 59 aa, synthetic construct
  REGION 1..59: note = Degron
NRTEAPEGTESEVETPSAINGNPSWQLADSPAINGATGHSSSLDAREVIPMAAVKQQAL

SEQ ID NO: 103 - protein, 37 aa, synthetic construct
  REGION 1..37: note = Degron
NRTEAPEGTESDMETPSAINGNASWHLADSPAVNGAT

SEQ ID NO: 104 - protein, 37 aa, synthetic construct
  REGION 1..37: note = Degron
NRTEAPEGTGPEMETPSAINGNPAWHPADSPAVNGAT

SEQ ID NO: 105 - protein, 37 aa, synthetic construct
  REGION 1..37: note = Degron
NRTEAPEGTESDMETPSAINGNPSWHLADSPAVNGAT

SEQ ID NO: 106 - protein, 37 aa, synthetic construct
  REGION 1..37: note = Degron
NRTEAPEGTESEAETPSAINGNPSWHLADSPAVNGAT

SEQ ID NO: 107 - protein, 37 aa, synthetic construct
  REGION 1..37: note = Degron
NRTEAPEGTESEMETPSAINGNPSWHLADSPPANGAT

SEQ ID NO: 108 - protein, 37 aa, synthetic construct
  REGION 1..37: note = Degron
NRTEAPEGTDSEMETPSAINGNPAWHLADSPAVNGAT

SEQ ID NO: 109 - protein, 37 aa, synthetic construct
  REGION 1..37: note = Degron
NRTEAPEGTDSEMETPSAINGNPSWHLADSPVVNGAT

SEQ ID NO: 110 - protein, 37 aa, synthetic construct
  REGION 1..37: note = Degron
NRTEAPEGTESEMETPSAINGNPSWHLADSPAVNGAT

SEQ ID NO: 111 - DNA, 21 bp, synthetic construct
  misc_feature 1..21: note = Degron1
  source 1..21: mol_type = other DNA
gcattggccccctacattcca

SEQ ID NO: 112 - DNA, 30 bp, synthetic construct
  misc_feature 1..30: note = Degron2
  source 1..30: mol_type = other DNA
gatcgccacgattcagggctcgattccatg